European Patent Application EP 4 585 684 A1, published July 16, 2025. Title: NUCLEIC ACIDS FOR TRANSFECTION. Applicant: AGC Inc. Application JP. The sequence listing filed with the application follows.

SEQUENCE LISTING (10 sequences)

SEQ ID NO: 1 - DNA, 22 bp, synthetic construct
  source 1..22: mol_type = other DNA
agggttagggttagggttaggg

SEQ ID NO: 2 - RNA, 21 nt, synthetic construct
  source 1..21: mol_type = other RNA
  misc_feature 20: note = dT
  misc_feature 21: note = dT
ggcgaagatcaacatggcatt

SEQ ID NO: 3 - RNA, 21 nt, synthetic construct
  source 1..21: mol_type = other RNA
  misc_feature 20: note = dT
  misc_feature 21: note = dT
tgccatgttgatcttcgcctt

SEQ ID NO: 4 - RNA, 21 nt, synthetic construct
  source 1..21: mol_type = other RNA
  misc_feature 20: note = dT
  misc_feature 21: note = dT
cggaagagtaactcacggatt

SEQ ID NO: 5 - RNA, 21 nt, synthetic construct
  source 1..21: mol_type = other RNA
  misc_feature 20: note = dT
  misc_feature 21: note = dT
tccgtgagttactcttccgtt

SEQ ID NO: 6 - RNA, 23 nt, synthetic construct
  source 1..23: mol_type = other RNA
cttacgctgagtacttcgaaatt

SEQ ID NO: 7 - RNA, 23 nt, synthetic construct
  source 1..23: mol_type = other RNA
tttcgaagtactcagcgtaagtt

SEQ ID NO: 8 - DNA, 19 bp, synthetic construct
  source 1..19: mol_type = other DNA
tttttcagttgaccatata

SEQ ID NO: 9 - RNA, 21 nt, synthetic construct
  source 1..21: mol_type = other RNA
  misc_feature 20: note = dT
  misc_feature 21: note = dT
tgcgctcctggacgtagcctt

SEQ ID NO: 10 - RNA, 21 nt, synthetic construct
  source 1..21: mol_type = other RNA
  misc_feature 20: note = dT
  misc_feature 21: note = dT
ggctacgtccaggagcgcatt